European Patent Specification EP 4 413 140 B1, published August 13, 2025. Title: Synthetic Genome Editing System. Applicant: Pencil Biosciences Limited. Application GB. The sequence listing filed with the application follows.

SEQUENCE LISTING (94 sequences)

SEQ ID NO: 1 - protein, 220 aa, synthetic construct
  REGION 1..220: note = ApGet polypeptide
MDAQTRRRERRAEKQAQWKAANGGGGSGGGGSGGGGSGGGGSGGGGSGGGGSGGGGSSLETWLKHREKDGGSGGGGSGGGGSGGGGGSIEKDIHINDGGIEIDIHIDSGGIEIDIHISSGSIEIDIHINNGNIEIDIHIGSDGIEIDIHIGNSGIEIDIHIDNGGIEIDIHIDSDGIEIDIHISSSGIEIDIHIGSEGIEIDIHIGDSGIEIDKHINQGS

SEQ ID NO: 2 - protein, 22 aa, synthetic construct
  REGION 1..22: note = RSBD corresponding to the Lambda N22 protein
MDAQTRRRERRAEKQAQWKAAN

SEQ ID NO: 3 - protein, 35 aa, synthetic construct
  REGION 1..35: note = linker
GGGGSGGGGSGGGGSGGGGSGGGGSGGGGSGGGGS

SEQ ID NO: 4 - protein, 15 aa, synthetic construct
  REGION 1..15: note = DBD
SLETWLKHREKDGGS

SEQ ID NO: 5 - protein, 16 aa, synthetic construct
  REGION 1..16: note = linker
GGGGSGGGGSGGGGGS

SEQ ID NO: 6 - protein, 132 aa, synthetic construct
  REGION 1..132: note = nuclease module
IEKDIHINDGGIEIDIHIDSGGIEIDIHISSGSIEIDIHINNGNIEIDIHIGSDGIEIDIHIGNSGIEIDIHIDNGGIEIDIHIDSDGIEIDIHISSSGIEIDIHIGSEGIEIDIHIGDSGIEIDKHINQGS

SEQ ID NO: 7 - protein, 7 aa, synthetic construct
  REGION 1..7: note = 7mer peptide unit
IEIDIHI

SEQ ID NO: 8 - protein, 7 aa, synthetic construct
  REGION 1..7: note = bD peptide
LELDLHL

SEQ ID NO: 9 - RNA, 24 nt, synthetic construct
  misc_feature 1..24: note = BoxB RNA scaffold
  source 1..24: mol_type = other RNA
aatttgggccctgaagaagggccc

SEQ ID NO: 10 - protein, 4 aa, synthetic construct
  REGION 1..4: note = 4mer tail sequence
NQGS

SEQ ID NO: 11 - protein, 4 aa, synthetic construct
  REGION 1..4: note = linker
NDGG

SEQ ID NO: 12 - protein, 4 aa, synthetic construct
  REGION 1..4: note = linker
DSSG

SEQ ID NO: 13 - protein, 4 aa, synthetic construct
  REGION 1..4: note = linker
SSGS

SEQ ID NO: 14 - protein, 4 aa, synthetic construct
  REGION 1..4: note = linker
NNGN

SEQ ID NO: 15 - protein, 4 aa, synthetic construct
  REGION 1..4: note = linker
GSDG

SEQ ID NO: 16 - protein, 4 aa, synthetic construct
  REGION 1..4: note = linker
GNSG

SEQ ID NO: 17 - protein, 4 aa, synthetic construct
  REGION 1..4: note = linker
DNGG

SEQ ID NO: 18 - protein, 4 aa, synthetic construct
  REGION 1..4: note = linker
DSDG

SEQ ID NO: 19 - protein, 4 aa, synthetic construct
  REGION 1..4: note = linker
SSSG

SEQ ID NO: 20 - protein, 4 aa, synthetic construct
  REGION 1..4: note = linker
GSEG

SEQ ID NO: 21 - protein, 4 aa, synthetic construct
  REGION 1..4: note = linker
GDSG

SEQ ID NO: 22 - protein, 7 aa, synthetic construct
  REGION 1..7: note = N-terminal flanking sequence
IEKDIHI

SEQ ID NO: 23 - protein, 7 aa, synthetic construct
  REGION 1..7: note = N-terminal flanking sequence
IEIDKHI

SEQ ID NO: 24 - protein, 11 aa, synthetic construct
  REGION 1..11: note = individual peptide unit
IEKDIHINDGG

SEQ ID NO: 25 - protein, 11 aa, synthetic construct
  REGION 1..11: note = individual peptide unit
IEIDIHIDSGG

SEQ ID NO: 26 - protein, 11 aa, synthetic construct
  REGION 1..11: note = individual peptide unit
IEIDIHISSGS

SEQ ID NO: 27 - protein, 11 aa, synthetic construct
  REGION 1..11: note = individual peptide unit
IEIDIHINNGN

SEQ ID NO: 28 - protein, 11 aa, synthetic construct
  REGION 1..11: note = individual peptide unit
IEIDIHIGSDG

SEQ ID NO: 29 - protein, 11 aa, synthetic construct
  REGION 1..11: note = individual peptide unit
IEIDIHIGNSG

SEQ ID NO: 30 - protein, 11 aa, synthetic construct
  REGION 1..11: note = individual peptide unit
IEIDIHIDNGG

SEQ ID NO: 31 - protein, 11 aa, synthetic construct
  REGION 1..11: note = individual peptide unit
IEIDIHIDSDG

SEQ ID NO: 32 - protein, 11 aa, synthetic construct
  REGION 1..11: note = individual peptide unit
IEIDIHISSSG

SEQ ID NO: 33 - protein, 11 aa, synthetic construct
  REGION 1..11: note = individual peptide unit
IEIDIHIGSEG

SEQ ID NO: 34 - protein, 11 aa, synthetic construct
  REGION 1..11: note = individual peptide unit
IEIDIHIGDSG

SEQ ID NO: 35 - protein, 11 aa, synthetic construct
  REGION 1..11: note = individual peptide unit
IEIDKHINQGS

SEQ ID NO: 36 - protein, 21 aa, synthetic construct
  REGION 1..21: note = anti-parallel beta sheet structure
  TURN 7..8: note = 4mer linker
  TURN 14..15: note = 4mer linker
IEIDIHIIEIDIHIIEIDIHI

SEQ ID NO: 37 - protein, 15 aa, synthetic construct
  REGION 1..15: note = Peptide 1
SLETWLKHREKDGGS

SEQ ID NO: 38 - protein, 12 aa, synthetic construct
  REGION 1..12: note = Peptide 2
SLETWLKHREKD

SEQ ID NO: 39 - protein, 15 aa, synthetic construct
  REGION 1..15: note = Peptide 3
AGDWESWTNGSWGGS

SEQ ID NO: 40 - protein, 12 aa, synthetic construct
  REGION 1..12: note = Peptide 4
AGDWESWTNGSW

SEQ ID NO: 41 - DNA, 21 bp, synthetic construct
  misc_feature 1..21: note = oligonucleotide 5
  misc_feature 21: note = TEG biotin
  source 1..21: mol_type = other DNA
  misc_feature 1..6: note = PDS
gaggtctttgttcttcttgtg

SEQ ID NO: 42 - DNA, 21 bp, synthetic construct
  misc_feature 1..21: note = oligonucleotide 6
  source 1..21: mol_type = other DNA
  misc_feature 16..21: note = PDS
cacaagaagaacaaagacctc

SEQ ID NO: 43 - DNA, 21 bp, synthetic construct
  misc_feature 1..21: note = oligonucleotide 7
  misc_feature 21: note = TEG biotin
  source 1..21: mol_type = other DNA
  misc_feature 1..6: note = PDS
acgggttttgttcttcttgtg

SEQ ID NO: 44 - DNA, 21 bp, synthetic construct
  misc_feature 1..21: note = oligonucleotide 8
  source 1..21: mol_type = other DNA
  misc_feature 16..21: note = PDS
cacaagaagaacaaaacccgt

SEQ ID NO: 45 - DNA, 21 bp, synthetic construct
  misc_feature 1..21: note = oligonucleotide 9
  misc_feature 21: note = TEG biotin
  source 1..21: mol_type = other DNA
atttcttgtgtgtgtaatgat

SEQ ID NO: 46 - DNA, 21 bp, synthetic construct
  misc_feature 1..21: note = oligonucleotide 10
  source 1..21: mol_type = other DNA
atcattacacacacaagaaat

SEQ ID NO: 47 - protein, 7 aa, synthetic construct
  REGION 1..7: note = bA peptide
LKLKLKL

SEQ ID NO: 48 - protein, 7 aa, synthetic construct
  REGION 1..7: note = bB peptide
LDLELHL

SEQ ID NO: 49 - protein, 7 aa, synthetic construct
  REGION 1..7: note = bC peptide
LDLDLHL

SEQ ID NO: 50 - protein, 9 aa, synthetic construct
  REGION 1..9: note = bE peptide
LDLDLELHL

SEQ ID NO: 51 - protein, 7 aa, synthetic construct
  REGION 1..7: note = bF peptide
IHIDIEL

SEQ ID NO: 52 - protein, 7 aa, synthetic construct
  REGION 1..7: note = bG peptide
IDIEIRI

SEQ ID NO: 53 - protein, 7 aa, synthetic construct
  REGION 1..7: note = bh peptide
IHIHIQI

SEQ ID NO: 54 - protein, 7 aa, synthetic construct
  REGION 1..7: note = bI peptide
LHLELNL

SEQ ID NO: 55 - protein, 7 aa, synthetic construct
  REGION 1..7: note = bJ peptide
LHLELHL

SEQ ID NO: 56 - protein, 7 aa, synthetic construct
  REGION 1..7: note = bK peptide
LNLYLEL

SEQ ID NO: 57 - protein, 9 aa, synthetic construct
  REGION 1..9: note = bL peptide
LDLDLKLHL

SEQ ID NO: 58 - protein, 7 aa, synthetic construct
  REGION 1..7: note = bM peptide
INIDIHL

SEQ ID NO: 59 - protein, 7 aa, synthetic construct
  REGION 1..7: note = bN peptide
IHIDISI

SEQ ID NO: 60 - DNA, 33 bp, synthetic construct
  misc_feature 1..33: note = DNA oligonucleotide
  misc_feature 1: note = 6-FAM
  misc_feature 33: note = BHQ1
  source 1..33: mol_type = other DNA
cctctccgtgtcttgtacttcccgtcagagagg

SEQ ID NO: 61 - DNA, 21 bp, synthetic construct
  misc_feature 1..21: note = target element sequence (TE) in the Editor plasmid
  source 1..21: mol_type = other DNA
gaactttcagtttagcggtct

SEQ ID NO: 62 - DNA, 246 bp, synthetic construct
  misc_feature 1..246: note = Target sequence in PC1 and PC2
  source 1..246: mol_type = other DNA
  misc_feature 1..21: note = Target sequence
  misc_feature 22..27: note = PDS
  misc_feature 67..87: note = Target sequence
  misc_feature 88..93: note = PDS
  misc_feature 133..153: note = Target sequence
  misc_feature 154..159: note = PDS
  misc_feature 199..219: note = Target Sequence
  misc_feature 220..225: note = PDS
gaactttcagtttagcggtctgaggtcccatagctgtttcctgtgtgatatcatgcagcggagtgcgaactttcagtttagcggtctgaggtcccatagctgtttcctgtgtgaatttcgcgcaacgcataagaactttcagtttagcggtctgaggtcccatagctgtttcctgtgtgatgcgccacatccacatcggaactttcagtttagcggtctgaggtcccatagctgtttcctgtgtga

SEQ ID NO: 63 - DNA, 21 bp, synthetic construct
  misc_feature 1..21: note = target element sequence
  source 1..21: mol_type = other DNA
cacacaggaaacagtattcat

SEQ ID NO: 64 - DNA, 54 bp, synthetic construct
  misc_feature 1..54: note = PDSout configuration
  source 1..54: mol_type = other DNA
  misc_feature 28..48: note = Target sequence
  misc_feature 49..54: note = PDS
gacctcatgaatactgtttcctgtgtgcacacaggaaacagtattcatgaggtc

SEQ ID NO: 65 - DNA, 59 bp, synthetic construct
  misc_feature 1..59: note = PDSin configuration with 5 nt spacer
  source 1..59: mol_type = other DNA
  misc_feature 1..21: note = Target sequence
  misc_feature 22..27: note = PDS
cacacaggaaacagtattcatgaggtcaattggacctcatgaatactgtttcctgtgtg

SEQ ID NO: 66 - DNA, 62 bp, synthetic construct
  misc_feature 1..62: note = PDSin configuration with 8 nt spacer
  source 1..62: mol_type = other DNA
  misc_feature 1..21: note = Target sequence
  misc_feature 22..27: note = PDS
cacacaggaaacagtattcatgaggtcaattggtcgacctcatgaatactgtttcctgtgtg

SEQ ID NO: 67 - DNA, 68 bp, synthetic construct
  misc_feature 1..68: note = PDSin configuration with 14 nt spacer
  source 1..68: mol_type = other DNA
  misc_feature 1..21: note = Target sequence
  misc_feature 22..27: note = PDS
cacacaggaaacagtattcatgaggtcgtttaaacgtcgacgacctcatgaatactgtttcctgtgtg

SEQ ID NO: 68 - DNA, 427 bp, synthetic construct
  misc_feature 1..427: note = Donor or repair template element
  source 1..427: mol_type = other DNA
  misc_feature 1..243: note = Left homology arm
  misc_feature 245..427: note = Right homology arm
gtacacggccgcataatcgaaattaatacgactcactataggggaattgtgagcggataacaattccccatcttagtatattagttaagtataagaaggagatatacatatggtgttcacactcgaagatttcgttggggactggcgacagacagccggctacaacctggaccaagtccttgaacagggaggtgtgtccagtttgtttcagaatctcggggtgtccgtaactccgatccaaaggattgtcctgagcggtgaaaatgggctgaagatcgacatccatgtcatcatcccgtatgaaggtctgagcggcgaccaaatgggccagatcgaaaaaatttttaaggtggtgtaccctgtggatgatcatcactttaaggtgatcctgcactatggcacactggtaatcgacggggttacgccg

SEQ ID NO: 69 - protein, 14 aa, synthetic construct
  REGION 1..14: note = L1a
EGKSSGSGSESKST

SEQ ID NO: 70 - protein, 30 aa, synthetic construct
  REGION 1..30: note = L2b
GGGGSGGGGSGGGGSGGGGSGGGGSGGGGS

SEQ ID NO: 71 - protein, 55 aa, synthetic construct
  REGION 1..55: note = VP64
GRADALDDFDLDMLGSDALDDFDLDMLGSDALDDFDLDMLGSDALDDFDLDMLIN

SEQ ID NO: 72 - DNA, 305 bp, synthetic construct
  source 1..305: mol_type = other DNA
  misc_feature 1..305: note = NAC1
  misc_feature 8..28: note = TE
  misc_feature 34..52: note = RS
aaaaaaatttattcagccgggagtccggaaattgggcccttcttcagggcccttacggtgtttcgtcctttccacaagatatataaagccaagaaatcgaaatactttcaagttacggtaagcatatgatagtccattttaaaacataattttaaaactgcaaactacccaagaaattattactttctacgtcacgtattttgtactaatatctttgtgtttacagtcaaattaattctaattatctctctaacagccttgtatcgtatatgcaaatatgaaggaatcatgggaaataggccctc

SEQ ID NO: 73 - DNA, 307 bp, synthetic construct
  source 1..307: mol_type = other DNA
  misc_feature 1..307: note = NAC2
  misc_feature 10..30: note = TE
  misc_feature 36..54: note = RS
aaaaaaaaagcgctttgcttcaagttcttaaaattgggcccttcttcagggcccttacggtgtttcgtcctttccacaagatatataaagccaagaaatcgaaatactttcaagttacggtaagcatatgatagtccattttaaaacataattttaaaactgcaaactacccaagaaattattactttctacgtcacgtattttgtactaatatctttgtgtttacagtcaaattaattctaattatctctctaacagccttgtatcgtatatgcaaatatgaaggaatcatgggaaataggccctc

SEQ ID NO: 74 - DNA, 305 bp, synthetic construct
  source 1..305: mol_type = other DNA
  misc_feature 1..305: note = NAC3
  misc_feature 254..272: note = RS
  misc_feature 278..298: note = TE
gagggcctatttcccatgattccttcatatttgcatatacgatacaaggctgttagagagataattagaattaatttgactgtaaacacaaagatattagtacaaaatacgtgacgtagaaagtaataatttcttgggtagtttgcagttttaaaattatgttttaaaatggactatcatatgcttaccgtaacttgaaagtatttcgatttcttggctttatatatcttgtggaaaggacgaaacaccgtaagggccctgaagaagggcccaatttgctccaatttctagggtcaccttttttt

SEQ ID NO: 75 - DNA, 305 bp, synthetic construct
  source 1..305: mol_type = other DNA
  misc_feature 1..305: note = NAC4
  misc_feature 254..272: note = RS
  misc_feature 284..298: note = TE
gagggcctatttcccatgattccttcatatttgcatatacgatacaaggctgttagagagataattagaattaatttgactgtaaacacaaagatattagtacaaaatacgtgacgtagaaagtaataatttcttgggtagtttgcagttttaaaattatgttttaaaatggactatcatatgcttaccgtaacttgaaagtatttcgatttcttggctttatatatcttgtggaaaggacgaaacaccgtaagggccctgaagaagggcccaatttggggctgggtgtcccattgaattttttt

SEQ ID NO: 76 - DNA, 2031 bp, synthetic construct
  source 1..2031: mol_type = other DNA
  misc_feature 1..2031: note = ApGeti-VP64
  misc_feature 1330..1395: note = RSBD DNA sequence
  misc_feature 1396..1500: note = Linker 2 DNA sequence
  misc_feature 1501..1545: note = DBD
  misc_feature 1546..1593: note = Linker 1 DNA sequence
  misc_feature 1594..1761: note = VP64 module DNA sequence
ggctccggtgcccgtcagtgggcagagcgcacatcgcccacagtccccgagaagttggggggaggggtcggcaattgaaccggtgcctagagaaggtggcgcggggtaaactgggaaagtgatgtcgtgtactggctccgcctttttcccgagggtgggggagaaccgtatataagtgcagtagtcgccgtgaacgttctttttcgcaacgggtttgccgccagaacacaggtaagtgccgtgtgtggttcccgcgggcctggcctctttacgggttatggcccttgcgtgccttgaattacttccacctggctgcagtacgtgattcttgatcccgagcttcgggttggaagtgggtgggagagttcgaggccttgcgcttaaggagccccttcgcctcgtgcttgagttgaggcctggcctgggcgctggggccgccgcgtgcgaatctggtggcaccttcgcgcctgtctcgctgctttcgataagtctctagccatttaaaatttttgatgacctgctgcgacgctttttttctggcaagatagtcttgtaaatgcgggccaagatctgcacactggtatttcggtttttggggccgcgggcggcgacggggcccgtgcgtcccagcgcacatgttcggcgaggcggggcctgcgagcgcggccaccgagaatcggacgggggtagtctcaagctggccggcctgctctggtgcctggcctcgcgccgccgtgtatcgccccgccctgggcggcaaggctggcccggtcggcaccagttgcgtgagcggaaagatggccgcttcccggccctgctgcagggagctcaaaatggaggacgcggcgctcgggagagcgggcgggtgagtcacccacacaaaggaaaagggcctttccgtcctcagccgtcgcttcatgtgactccacggagtaccgggcgccgtccaggcacctcgattagttctcgagcttttggagtacgtcgtctttaggttggggggaggggttttatgcgatggagtttccccacactgagtgggtggagactgaagttaggccagcttggcacttgatgtaattctccttggaatttgccctttttgagtttggatcttggttcattctcaagcctcagacagtggttcaaagtttttttcttccatttcaggtgtcgtgacaagtttgtacaaaaaagcaggctgccaccatggactataaggaccacgacggagactacaaggatcatgatattgattacaaagacgatgacgataagatggccccaaagaagaagcggaaggtcggtatccacggagtcccagcagctatggacgctcagacaagaagaagagagcgtcgggccgaaaagcaagctcagtggaaggcggcgaatggaggtggcggatcgggcggcggcgggagcggtggtggtggcagcggcggtggcggaagcggaggaggggggagcggcggcggaggtagcggagggggggggtcctccctggaaacctggctgaaacacagagagaaggacggtgggagtggtggtggagggagcggcggaggtggcagcggcggcgggggcgggtcaggacgggctgacgcattggacgattttgatctggatatgctgggaagtgacgccctcgatgattttgaccttgacatgcttggttcggatgcccttgatgactttgacctcgacatgctcggcagtgacgcccttgatgatttcgacctggacatgctgattaactgacagcacccagctttcttgtacaaagtggtgatggccggccgcttcgagcagacatgataagatacattgatgagtttggacaaaccacaactagaatgcagtgaaaaaaatgctttatttgtgaaatttgtgatgctattgctttatttgtaaccattataagctgcaataaacaagttaacaacaacaattgcattcattttatgtttcaggttcagggggaggtgtgggaggttttttaaagcaagtaaaacctctacaaatgtggta

SEQ ID NO: 77 - DNA, 66 bp, synthetic construct
  source 1..66: mol_type = other DNA
  misc_feature 1..66: note = RSBD (Lambda N22) DNA sequence
atggacgctcagacaagaagaagagagcgtcgggccgaaaagcaagctcagtggaaggcggcgaat

SEQ ID NO: 78 - DNA, 48 bp, synthetic construct
  source 1..48: mol_type = other DNA
  misc_feature 1..48: note = Linker 1 (L1) DNA sequence
ggtggtggagggagcggcggaggtggcagcggcggcgggggcgggtca

SEQ ID NO: 79 - DNA, 42 bp, synthetic construct
  source 1..42: mol_type = other DNA
  misc_feature 1..42: note = Modified linker 1 (L1a) DNA sequence
gagggaaaatcttccgggagtggttcagaatctaagagcacc

SEQ ID NO: 80 - DNA, 105 bp, synthetic construct
  source 1..105: mol_type = other DNA
  misc_feature 1..105: note = Linker 2 (L2) DNA sequence
ggaggtggcggatcgggcggcggcgggagcggtggtggtggcagcggcggtggcggaagcggaggaggggggagcggcggcggaggtagcggagggggggggtcc

SEQ ID NO: 81 - DNA, 90 bp, synthetic construct
  source 1..90: mol_type = other DNA
  misc_feature 1..90: note = Modified linker 2 (L2b) DNA sequence
ggcggcggcgggagcggtggtggtggcagcggcggtggcggaagcggaggaggggggagcggcggcggaggtagcggagggggggggtcc

SEQ ID NO: 82 - DNA, 168 bp, synthetic construct
  source 1..168: mol_type = other DNA
  misc_feature 1..168: note = VP64 module DNA sequence
ggacgggctgacgcattggacgattttgatctggatatgctgggaagtgacgccctcgatgattttgaccttgacatgcttggttcggatgcccttgatgactttgacctcgacatgctcggcagtgacgcccttgatgatttcgacctggacatgctgattaactga

SEQ ID NO: 83 - DNA, 45 bp, synthetic construct
  source 1..45: mol_type = other DNA
  misc_feature 1..45: note = DBD DNA sequence
tccctggaaacctggctgaaacacagagagaaggacggtgggagt

SEQ ID NO: 84 - DNA, 300 bp, synthetic construct
  source 1..300: mol_type = other DNA
  misc_feature 1..300: note = Detector plasmid sequence
  misc_feature 157..162: note = PDS
  misc_feature 163..183: note = Target
  misc_feature 43..65: note = CAP binding site
  misc_feature 80..108: note = lac promoter
  misc_feature 117..133: note = lac operator
  misc_feature 195..300: note = Nluc
caggtttgccgactggaaagcgggcagtgagcgcaacgcaattaatgtgagttagctcactcattaggcaccccaggctttacactttatgcttccggctcgtatgttgtgtggaattgtgagcggataacaatttcacacaggaaacagctatggtacctcacaccgctaaactgaaagttcgtggtggcagcatggtgttcacactcgaagatttcgttggggactggcgacagacagccggctacaacctggaccaagtccttgaacagggaggtgtgtccagtttgtttcagaatc

SEQ ID NO: 85 - DNA, 500 bp, synthetic construct
  source 1..500: mol_type = other DNA
  misc_feature 1..500: note = Fragment of the PD-L1 gene sequence
  misc_feature 209..214: note = PDS
  misc_feature 215..235: note = PD-L target
  misc_feature 236..256: note = PD-L target
  misc_feature 257..262: note = PDS
  misc_feature 132..419: note = CD274-001 Exon 4
catctgaacattaagcatatccctctgagaaccagcctgcattgatactctttctaatgtggacagcatcaagctatgtacgtagttctgtgctcagcaaaagccctgacttctttttgtttatgtcctagccccatacaacaaaatcaaccaaagaattttggttgtggatccagtcacctctgaacatgaactgacatgtcaggctgagggctaccccaaggccgaagtcatctggacaagcagtgaccatcaagtcctgagtggtaagaccaccaccaccaattccaagagagaggagaagcttttcaatgtgaccagcacactgagaatcaacacaacaactaatgagattttctactgcacttttaggagattagatcctgaggaaaaccatacagctgaattggtcatcccaggtaatattctgaatgtgtccattaaaatatgtctaacactgtcccctagcacctagcatgatgtctgcctatcatagtcat

SEQ ID NO: 86 - DNA, 456 bp, synthetic construct
  source 1..456: mol_type = other DNA
  misc_feature 1..456: note = Genomic reference sequence
  misc_feature 16..35: note = Fp3
  misc_feature 154..159: note = PDS
  misc_feature 160..180: note = T3
  misc_feature 187..207: note = T4
  misc_feature 208..213: note = PDS
  misc_feature 368..387: note = Rp3
aacctgctcaccagcatctcacccactgccttctcccgccttcgctacctggagtcgcttgacctcagccacaatggcctgacagccctgccagccgagagcttcaccagctcacccctgagcgacgtgaaccttagccacaaccagctccgggaggtctcagtgtctgccttcacgacgcacagtcagggccgggcactacacttggacctctcccacaacctcattcaccgcctcgtgccccaccccacgagggccggcctgcctgcgcccaccattcagagcctgaacctggcctggaaccggctccatgccgtgcccaacctccgagacttgcccctgcgctacctgagcctggatgggaaccctctagctgtcattggtccgggtgccttcgcggggctgggaggccttacacacctgtctctggccagcctgcagaggctccctgagctg

SEQ ID NO: 87 - DNA, 100 bp, synthetic construct
  source 1..100: mol_type = other DNA
  misc_feature 1..100: note = Sanger sequencing of wild-type sequence
aaccagctccgggaggtctcagtgtctgccttcacgacgcacagtcagggccgggcactacacttggacctctcccacaacctcattcaccgcctcgtgc

SEQ ID NO: 88 - DNA, 100 bp, synthetic construct
  source 1..100: mol_type = other DNA
  misc_feature 1..100: note = Sanger sequencing of ApGet transfected samples
  unsure 5..6
  unsure 11
  unsure 13
  unsure 15
  unsure 22
  unsure 39
  unsure 42
  unsure 44
  unsure 47
  unsure 51
  unsure 53
  unsure 55
  unsure 62
  unsure 67
  unsure 79
aaccnnctccngnangtctcantgtctgccttcacgacncanantcngggncngncactacncttgnacctctcccacnacctcattcaccgcctcgtgc

SEQ ID NO: 89 - protein, 5 aa, synthetic construct
  REGION 1..5: note = Suitable linker
  REGION 1..5: note = Sequence repeated n times
GGGGS

SEQ ID NO: 90 - protein, 15 aa, synthetic construct
  REGION 1..15: note = Non-inverted multimer
  REGION 1..15: note = Sequence repeated n times
  REGION 8: note = X repeated n times
  REGION 8: note = X represents a linker
  REGION 2: note = X: represents catalytic amino acid C1
  REGION 4: note = X: represents catalytic amino acid C2
  REGION 6: note = X: represents catalytic amino acid C3
  REGION 10: note = X: represents catalytic amino acid C1
  REGION 12: note = X: represents catalytic amino acid C2
  REGION 14: note = X: represents catalytic amino acid C3
  REGION 1: note = H: a hydrophobic residue, preferably leucine or isoleucine, most preferably isoleucine
  REGION 3: note = H: a hydrophobic residue, preferably leucine or isoleucine, most preferably isoleucine
  REGION 5: note = H: a hydrophobic residue, preferably leucine or isoleucine, most preferably isoleucine
  REGION 7: note = H: a hydrophobic residue, preferably leucine or isoleucine, most preferably isoleucine
  REGION 9: note = H: a hydrophobic residue, preferably leucine or isoleucine, most preferably isoleucine
  REGION 11: note = H: a hydrophobic residue, preferably leucine or isoleucine, most preferably isoleucine
  REGION 13: note = H: a hydrophobic residue, preferably leucine or isoleucine, most preferably isoleucine
  REGION 15: note = H: a hydrophobic residue, preferably leucine or isoleucine, most preferably isoleucine
HXHXHXHXHXHXHXH

SEQ ID NO: 91 - protein, 15 aa, synthetic construct
  REGION 1..15: note = Inverted multimer
  REGION 8: note = X represents a linker
  REGION 8: note = X repeated n times
  REGION 1..15: note = Sequence repeated n times
  REGION 1: note = H: a hydrophobic residue, preferably leucine or isoleucine, most preferably isoleucine
  REGION 3: note = H: a hydrophobic residue, preferably leucine or isoleucine, most preferably isoleucine
  REGION 5: note = H: a hydrophobic residue, preferably leucine or isoleucine, most preferably isoleucine
  REGION 7: note = H: a hydrophobic residue, preferably leucine or isoleucine, most preferably isoleucine
  REGION 9: note = H: a hydrophobic residue, preferably leucine or isoleucine, most preferably isoleucine
  REGION 11: note = H: a hydrophobic residue, preferably leucine or isoleucine, most preferably isoleucine
  REGION 13: note = H: a hydrophobic residue, preferably leucine or isoleucine, most preferably isoleucine
  REGION 15: note = H: a hydrophobic residue, preferably leucine or isoleucine, most preferably isoleucine
  REGION 2: note = X: represents catalytic amino acid C1
  REGION 4: note = X: represents catalytic amino acid C2
  REGION 6: note = X: represents catalytic amino acid C3
  REGION 10: note = X: represents catalytic amino acid C3
  REGION 12: note = X: represents catalytic amino acid C2
  REGION 14: note = X: represents catalytic amino acid C1
HXHXHXHXHXHXHXH

SEQ ID NO: 92 - protein, 49 aa, synthetic construct
  REGION 1..7: note = Negative design peptide unit
  REGION 1: note = H: a hydrophobic residue
  REGION 5: note = H: a hydrophobic residue
  REGION 7: note = H: a hydrophobic residue
  REGION 2: note = X: a catalytic residue
  REGION 4: note = X: a catalytic residue
  REGION 6: note = X: a catalytic residue
  REGION 1..49: note = ApGET1.0: Pentamer
  REGION 43..49: note = Negative design peptide unit
  REGION 8: note = H: a hydrophobic residue
  REGION 10: note = H: a hydrophobic residue
  REGION 12: note = H: a hydrophobic residue
  REGION 14: note = H: a hydrophobic residue
  REGION 15: note = H: a hydrophobic residue
  REGION 17: note = H: a hydrophobic residue
  REGION 19: note = H: a hydrophobic residue
  REGION 21: note = H: a hydrophobic residue
  REGION 22: note = H: a hydrophobic residue
  REGION 24: note = H: a hydrophobic residue
  REGION 26: note = H: a hydrophobic residue
  REGION 28: note = H: a hydrophobic residue
  REGION 29: note = H: a hydrophobic residue
  REGION 31: note = H: a hydrophobic residue
  REGION 33: note = H: a hydrophobic residue
  REGION 35: note = H: a hydrophobic residue
  REGION 36: note = H: a hydrophobic residue
  REGION 38: note = H: a hydrophobic residue
  REGION 40: note = H: a hydrophobic residue
  REGION 42: note = H: a hydrophobic residue
  REGION 43: note = H: a hydrophobic residue
  REGION 45: note = H: a hydrophobic residue
  REGION 49: note = H: a hydrophobic residue
  TURN 7..8: note = 4 amino acid beta turn
  TURN 14..15: note = 4 amino acid beta turn
  TURN 21..22: note = 4 amino acid beta turn
  TURN 28..29: note = 4 amino acid beta turn
  TURN 35..36: note = 4 amino acid beta turn
  TURN 42..43: note = 4 amino acid beta turn
  REGION 9: note = X: a catalytic residue
  REGION 11: note = X: a catalytic residue
  REGION 13: note = X: a catalytic residue
  REGION 16: note = X: a catalytic residue
  REGION 18: note = X: a catalytic residue
  REGION 20: note = X: a catalytic residue
  REGION 23: note = X: a catalytic residue
  REGION 25: note = X: a catalytic residue
  REGION 27: note = X: a catalytic residue
  REGION 30: note = X: a catalytic residue
  REGION 32: note = X: a catalytic residue
  REGION 34: note = X: a catalytic residue
  REGION 37: note = X: a catalytic residue
  REGION 39: note = X: a catalytic residue
  REGION 41: note = X: a catalytic residue
  REGION 44: note = X: a catalytic residue
  REGION 46: note = X: a catalytic residue
  REGION 48: note = X: a catalytic residue
HXKXHXHHXHXHXHHXHXHXHHXHXHXHHXHXHXHHXHXHXHHXHXKXH

SEQ ID NO: 93 - protein, 84 aa, synthetic construct
  REGION 1..84: note = ApGET1.0: Decamer
  TURN 7..8: note = 4 amino acid beta turn
  TURN 14..15: note = 4 amino acid beta turn
  TURN 21..22: note = 4 amino acid beta turn
  TURN 28..29: note = 4 amino acid beta turn
  TURN 35..36: note = 4 amino acid beta turn
  TURN 42..43: note = 4 amino acid beta turn
  TURN 49..50: note = 4 amino acid beta turn
  TURN 56..57: note = 4 amino acid beta turn
  TURN 63..64: note = 4 amino acid beta turn
  TURN 70..71: note = 4 amino acid beta turn
  TURN 77..78: note = 4 amino acid beta turn
  REGION 1: note = H: a hydrophobic residue
  REGION 5: note = H: a hydrophobic residue
  REGION 7: note = H: a hydrophobic residue
  REGION 8: note = H: a hydrophobic residue
  REGION 10: note = H: a hydrophobic residue
  REGION 12: note = H: a hydrophobic residue
  REGION 14: note = H: a hydrophobic residue
  REGION 15: note = H: a hydrophobic residue
  REGION 17: note = H: a hydrophobic residue
  REGION 19: note = H: a hydrophobic residue
  REGION 21: note = H: a hydrophobic residue
  REGION 22: note = H: a hydrophobic residue
  REGION 24: note = H: a hydrophobic residue
  REGION 26: note = H: a hydrophobic residue
  REGION 28: note = H: a hydrophobic residue
  REGION 29: note = H: a hydrophobic residue
  REGION 31: note = H: a hydrophobic residue
  REGION 33: note = H: a hydrophobic residue
  REGION 35: note = H: a hydrophobic residue
  REGION 36: note = H: a hydrophobic residue
  REGION 38: note = H: a hydrophobic residue
  REGION 40: note = H: a hydrophobic residue
  REGION 42: note = H: a hydrophobic residue
  REGION 43: note = H: a hydrophobic residue
  REGION 45: note = H: a hydrophobic residue
  REGION 47: note = H: a hydrophobic residue
  REGION 49: note = H: a hydrophobic residue
  REGION 50: note = H: a hydrophobic residue
  REGION 52: note = H: a hydrophobic residue
  REGION 54: note = H: a hydrophobic residue
  REGION 56: note = H: a hydrophobic residue
  REGION 57: note = H: a hydrophobic residue
  REGION 59: note = H: a hydrophobic residue
  REGION 61: note = H: a hydrophobic residue
  REGION 63: note = H: a hydrophobic residue
  REGION 64: note = H: a hydrophobic residue
  REGION 66: note = H: a hydrophobic residue
  REGION 68: note = H: a hydrophobic residue
  REGION 70: note = H: a hydrophobic residue
  REGION 71: note = H: a hydrophobic residue
  REGION 73: note = H: a hydrophobic residue
  REGION 75: note = H: a hydrophobic residue
  REGION 77: note = H: a hydrophobic residue
  REGION 78: note = H: a hydrophobic residue
  REGION 80: note = H: a hydrophobic residue
  REGION 84: note = H: a hydrophobic residue
  REGION 2: note = X: a catalytic residue
  REGION 4: note = X: a catalytic residue
  REGION 6: note = X: a catalytic residue
  REGION 9: note = X: a catalytic residue
  REGION 11: note = X: a catalytic residue
  REGION 13: note = X: a catalytic residue
  REGION 16: note = X: a catalytic residue
  REGION 18: note = X: a catalytic residue
  REGION 20: note = X: a catalytic residue
  REGION 23: note = X: a catalytic residue
  REGION 25: note = X: a catalytic residue
  REGION 27: note = X: a catalytic residue
  REGION 30: note = X: a catalytic residue
  REGION 32: note = X: a catalytic residue
  REGION 34: note = X: a catalytic residue
  REGION 37: note = X: a catalytic residue
  REGION 39: note = X: a catalytic residue
  REGION 41: note = X: a catalytic residue
  REGION 44: note = X: a catalytic residue
  REGION 46: note = X: a catalytic residue
  REGION 48: note = X: a catalytic residue
  REGION 51: note = X: a catalytic residue
  REGION 53: note = X: a catalytic residue
  REGION 55: note = X: a catalytic residue
  REGION 58: note = X: a catalytic residue
  REGION 60: note = X: a catalytic residue
  REGION 62: note = X: a catalytic residue
  REGION 65: note = X: a catalytic residue
  REGION 67: note = X: a catalytic residue
  REGION 69: note = X: a catalytic residue
  REGION 72: note = X: a catalytic residue
  REGION 74: note = X: a catalytic residue
  REGION 76: note = X: a catalytic residue
  REGION 79: note = X: a catalytic residue
  REGION 81: note = X: a catalytic residue
  REGION 83: note = X: a catalytic residue
  REGION 1..7: note = Negative design peptide unit
  REGION 78..84: note = Negative design peptide unit
HXKXHXHHXHXHXHHXHXHXHHXHXHXHHXHXHXHHXHXHXHHXHXHXHHXHXHXHHXHXHXHHXHXHXHHXHXHXHHXHXKXH

SEQ ID NO: 94 - protein, 35 aa, synthetic construct
  REGION 1..35: note = Nluc
MVFTLEDFVGDWRQTAGYNLDQVLEQGGVSSLFQN